European Patent Application EP 4 445 954 A2, published October 16, 2024. Title: CELLULAR MODELS OF AND THERAPIES FOR OCULAR DISEASES. Applicant: Reflection Biotechnologies Limited. Application EP, filed July 31, 2018. The sequence listing filed with the application follows.

SEQUENCE LISTING (64 sequences)

SEQ ID NO: 1 - DNA, 1578 bp, synthetic construct
  misc_feature 1..1578: note = Synthetically generated coding sequence
  source 1..1578: mol_type = other DNA
atggcggggctctggctggggctcgtgtggcagaagctgctgctgtggggcgcggcgagtgccctttccctggccggcgccagtctggtcctgagcctgctgcagagggtggcgagctacgcgcggaaatggcagcagatgcggcccatccccacggtggcccgcgcctacccactggtgggccacgcgctgctgatgaagccggacgggcgagaattttttcagcagatcattgagtacacagaggaataccgccacatgccgctgctgaagctctgggtcgggccagtgcccatggtggccctttataatgcagaaaatgtggaggtaattttaactagttcaaagcaaattgacaaatcctctatgtacaagtttttagaaccatggcttggcctaggacttcttacaagtactggaaacaaatggcgctccaggagaaagatgttaacacccactttccattttaccattctggaagatttcttagatatcatgaatgaacaagcaaatatattggttaagaaacttgaaaaacacattaaccaagaagcatttaactgctttttttacatcactctttgtgccttagatatcatctgtgaaacagctatggggaagaatattggtgctcaaagtaatgatgattccgagtatgtccgtgcagtttatagaatgagtgagatgatatttcgaagaataaagatgccctggctttggcttgatctctggtaccttatgtttaaagaaggatgggaacacaaaaagagccttcagatcctacatacttttaccaacagtgtcatcgctgaacgggccaatgaaatgaacgccaatgaagactgtagaggtgatggcaggggctctgccccctccaaaaataaacgcagggcctttcttgacttgcttttaagtgtgactgatgacgaagggaacaggctaagtcatgaagatattcgagaagaagttgacaccttcatgtttgaggggcacgatacaactgcagctgcaataaactggtccttatacctgttgggttctaacccagaagtccagaaaaaagtggatcatgaattggatgacgtgtttgggaagtctgaccgtcccgctacagtagaagacctgaagaaacttcggtatctggaatgtgttattaaggagacccttcgcctttttccttctgttcctttatttgcccgtagtgttagtgaagattgtgaagtggcaggttacagagttctaaaaggcactgaagccgtcatcattccctatgcattgcacagagatccgagatacttccccaaccccgaggagttccagcctgagcggttcttccccgagaatgcacaagggcgccatccatatgcctacgtgcccttctctgctggccccaggaactgtataggtcaaaagtttgctgtgatggaagaaaagaccattctttcgtgcatcctgaggcacttttggatagaatccaaccagaaaagagaagagcttggtctagaaggacagttgattcttcgtccaagtaatggcatctggatcaagttgaagaggagaaatgcagatgaacgctaa

SEQ ID NO: 2 - DNA, 1578 bp, synthetic construct
  misc_feature 1..1578: note = Synthetically generated coding sequence
  source 1..1578: mol_type = other DNA
atggctggactgtggctgggactggtgtggcagaaactgctgctgtggggggccgcttccgcactgtcactggctggggcttcactggtgctgagcctgctgcagagggtggcctcctacgccagaaagtggcagcagatgaggcccatccctaccgtggccagagcctatccactggtgggacacgcactgctgatgaagcctgacggcagagagttctttcagcagatcatcgagtacacagaggagtataggcacatgccactgctgaagctgtgggtgggacccgtgcctatggtggccctgtacaacgccgagaatgtggaagtgatcctgaccagcagcaagcagatcgataagtctagcatgtataagttcctggagccttggctgggcctgggcctgctgacctctacaggcaacaagtggaggagccggagaaagatgctgaccccaacattccactttacaatcctggaggacttcctggacatcatgaacgagcaggccaatatcctggtgaagaagctggagaagcacatcaaccaggaggcctttaattgcttcttttacatcaccctgtgcgccctggacatcatctgtgagacagctatgggcaagaacatcggcgcccagtctaatgacgatagcgagtacgtgcgggccgtgtatagaatgagcgagatgatctttaggcgcatcaagatgccctggctgtggctggatctgtggtatctgatgttcaaggagggctgggagcacaagaagtccctgcagatcctgcacacctttacaaactctgtgatcgccgagagagccaatgagatgaacgccaatgaggactgtaggggcgatggaaggggcagcgccccttccaagaacaagcggagagccttcctggacctgctgctgagcgtgaccgacgatgagggcaatcgcctgtcccacgaggacatccgggaggaggtggatacattcatgtttgagggacacgacaccacagccgccgccatcaactggtccctgtacctgctgggctctaatccagaggtgcagaagaaggtggatcacgagctggacgacgtgttcggcaagtccgacaggccagcaaccgtggaggatctgaagaagctgagatacctggagtgcgtgatcaaggagacactgcgcctgttcccctctgtgcctctgtttgcccggtccgtgtctgaggactgtgaggtggccggctatcgcgtgctgaagggcaccgaggccgtgatcatcccttacgccctgcaccgggaccccaggtatttccctaacccagaggagtttcagccagagagattctttcccgagaatgcccagggcaggcacccttacgcctatgtgccattctccgccggaccaaggaactgcatcggacagaagtttgccgtgatggaggagaaaaccatcctgtcttgtatcctgagacacttctggatcgagagcaatcagaagagggaggagctgggcctggagggacagctgatcctgcggccaagcaacggcatctggatcaaactgaaaagaaggaacgctgacgagaggtaa

SEQ ID NO: 3 - DNA, 1578 bp, synthetic construct
  misc_feature 1..1578: note = Synthetically generated coding sequence
  source 1..1578: mol_type = other DNA
atggcggggctctggctggggctcgtgtggcagaagctgctgctgtggggcgcggcgagtgccctttccctggccggcgccagtctggtcctgagcctgctgcagagggtggcgagctacgcgcggaaatggcagcagatgcggcccatccccacggtggcccgcgcctacccactggtgggccacgcgctgctgatgaagccggacgggcgagaattttttcagcagatcattgagtacacagaggaataccgccacatgccgctgctgaagctctgggtcgggccagtgcccatggtggccctttataatgcagaaaatgtggaggtaattttaactagttcaaagcaaattgacaaatcctctatgtacaagtttttagaaccatggcttggcctaggacttcttacaagtactggaaacaaatggcgctccaggagaaagatgttaacacccactttccattttaccattctggaagatttcttagatatcatgaatgaacaagcaaatatattggttaagaaacttgaaaaacacattaaccaagaagcatttaactgctttttttacatcactctttgtgccttagatatcatctgtgaaacagctatggggaagaatattggtgctcaaagtaatgatgattccgagtatgtccgtgcagtttatagaatgagtgagatgatatttcgaagaataaagatgccctggctttggcttgatctctggtaccttatgtttaaagaaggatgggaacacaaaaagagccttaagatcctacatacttttaccaacagtgtcatcgcggaacgggccaatgaaatgaacgccaatgaagactgtagaggtgatggcaggggctctgccccctccaaaaataaacgcagggcctttcttgacttgcttttaagtgtgactgatgacgaagggaacaggctaagtcatgaagatattcgagaagaagttgacaccttcatgtttgaggggcacgatacaactgcagctgcaataaactggtccttatacctgttgggttctaacccagaagtccagaaaaaagtggatcatgaattggatgacgtgtttgggaagtctgaccgtcccgctacagtagaagacctgaagaaacttcggtatctggaatgtgttattaaggagacccttcgcctttttccttctgttcctttatttgcccgtagtgttagtgaagattgtgaagtggcaggttacagagttctaaaaggcactgaagccgtcatcattccctatgcattgcacagagatccgagatacttccccaaccccgaggagttccagcctgagcggttcttccccgagaatgcacaagggcgccatccatatgcctacgtgcccttctctgctggccccaggaactgtataggtcaaaagtttgctgtgatggaagaaaagaccattctttcgtgcatcctgaggcacttttggatagaatccaaccagaaaagagaagagcttggtctagaaggacagttgattcttcgtccaagtaatggcatctggatcaagttgaagaggagaaatgcagatgaacgctaa

SEQ ID NO: 4 - protein, 525 aa, Homo sapiens
MAGLWLGLVWQKLLLWGAASALSLAGASLVLSLLQRVASYARKWQQMRPIPTVARAYPLVGHALLMKPDGREFFQQIIEYTEEYRHMPLLKLWVGPVPMVALYNAENVEVILTSSKQIDKSSMYKFLEPWLGLGLLTSTGNKWRSRRKMLTPTFHFTILEDFLDIMNEQANILVKKLEKHINQEAFNCFFYITLCALDIICETAMGKNIGAQSNDDSEYVRAVYRMSEMIFRRIKMPWLWLDLWYLMFKEGWEHKKSLQILHTFTNSVIAERANEMNANEDCRGDGRGSAPSKNKRRAFLDLLLSVTDDEGNRLSHEDIREEVDTFMFEGHDTTAAAINWSLYLLGSNPEVQKKVDHELDDVFGKSDRPATVEDLKKLRYLECVIKETLRLFPSVPLFARSVSEDCEVAGYRVLKGTEAVIIPYALHRDPRYFPNPEEFQPERFFPENAQGRHPYAYVPFSAGPRNCIGQKFAVMEEKTILSCILRHFWIESNQKREELGLEGQLILRPSNGIWIKLKRRNADER

SEQ ID NO: 5 - protein, 525 aa, Homo sapiens
MAGLWLGLVWQKLLLWGAASALSLAGASLVLSLLQRVASYARKWQQMRPIPTVARAYPLVGHALLMKPDGREFFQQIIEYTEEYRHMPLLKLWVGPVPMVALYNAENVEVILTSSKQIDKSSMYKFLEPWLGLGLLTSTGNKWRSRRKMLTPTFHFTILEDFLDIMNEQANILVKKLEKHINQEAFNCFFYITLCALDIICETAMGKNIGAQSNDDSEYVRAVYRMSEMIFRRIKMPWLWLDLWYLMFKEGWEHKKSLKILHTFTNSVIAERANEMNANEDCRGDGRGSAPSKNKRRAFLDLLLSVTDDEGNRLSHEDIREEVDTFMFEGHDTTAAAINWSLYLLGSNPEVQKKVDHELDDVFGKSDRPATVEDLKKLRYLECVIKETLRLFPSVPLFARSVSEDCEVAGYRVLKGTEAVIIPYALHRDPRYFPNPEEFQPERFFPENAQGRHPYAYVPFSAGPRNCIGQKFAVMEEKTILSCILRHFWIESNQKREELGLEGQLILRPSNGIWIKLKRRNADER

SEQ ID NO: 6 - protein, 490 aa, Homo sapiens
RVASYARKWQQMRPIPTVARAYPLVGHALLMKPDGREFFQQIIEYTEEYRHMPLLKLWVGPVPMVALYNAENVEVILTSSKQIDKSSMYKFLEPWLGLGLLTSTGNKWRSRRKMLTPTFHFTILEDFLDIMNEQANILVKKLEKHINQEAFNCFFYITLCALDIICETAMGKNIGAQSNDDSEYVRAVYRMSEMIFRRIKMPWLWLDLWYLMFKEGWEHKKSLQILHTFTNSVIAERANEMNANEDCRGDGRGSAPSKNKRRAFLDLLLSVTDDEGNRLSHEDIREEVDTFMFEGHDTTAAAINWSLYLLGSNPEVQKKVDHELDDVFGKSDRPATVEDLKKLRYLECVIKETLRLFPSVPLFARSVSEDCEVAGYRVLKGTEAVIIPYALHRDPRYFPNPEEFQPERFFPENAQGRHPYAYVPFSAGPRNCIGQKFAVMEEKTILSCILRHFWIESNQKREELGLEGQLILRPSNGIWIKLKRRNADER

SEQ ID NO: 7 - protein, 500 aa, Homo sapiens
MSPGLLLLGSAVLLAFGLCCTFVHRARSRYEHIPGPPRPSFLLGHLPCFWKKDEVGGRVLQDVFLDWAKKYGPVVRVNVFHKTSVIVTSPESVKKFLMSTKYNKDSKMYRALQTVFGERLFGQGLVSECNYERWHKQRRVIDLAFSRSSLVSLMETFNEKAEQLVEILEAKADGQTPVSMQDMLTYTAMDILAKAAFGMETSMLLGAQKPLSQAVKLMLEGITASRNTLAKFLPGKRKQLREVRESIRFLRQVGRDWVQRRREALKRGEEVPADILTQILKAEEGAQDDEGLLDNFVTFFIAGHETSANHLAFTVMELSRQPEIVARLQAEVDEVIGSKRYLDFEDLGRLQYLSQVLKESLRLYPPAWGTFRLLEEETLIDGVRVPGNTPLLFSTYVMGRMDTYFEDPLTFNPDRFGPGAPKPRFTYFPFSLGHRSCIGQQFAQMEVKVVMAKLLQRLEFRLVPGQRFGLQEQATLKPLDPVLCTLRPRGWQPAPPPPPC

SEQ ID NO: 8 - protein, 519 aa, Homo sapiens
MSVSVLSPSRLLGDVSGILQAASLLILLLLLIKAVQLYLHRQWLLKALQQFPCPPSHWLFGHIQELQQDQELQRIQKWVETFPSACPHWLWGGKVRVQLYDPDYMKVILGRSDPKSHGSYRFLAPWIGYGLLLLNGQTWFQHRRMLTPAFHYDILKPYVGLMADSVRVMLDKWEELLGQDSPLEVFQHVSLMTLDTIMKCAFSHQGSIQVDRNSQSYIQAISDLNNLVFSRVRNAFHQNDTIYSLTSAGRWTHRACQLAHQHTDQVIQLRKAQLQKEGELEKIKRKRHLDFLDILLLAKMENGSILSDKDLRAEVDTFMFEGHDTTASGISWILYALATHPKHQERCREEIHSLLGDGASITWNHLDQMPYTTMCIKEALRLYPPVPGIGRELSTPVTFPDGRSLPKGIMVLLSIYGLHHNPKVWPNPEVFDPFRFAPGSAQHSHAFLPFSGGSRNCIGKQFAMNELKVATALTLLRFELLPDPTRIPIPIARLVLKSKNGIHLRLRRLPNPCEDKDQL

SEQ ID NO: 9 - protein, 519 aa, Homo sapiens
MSVSVLSPSRRLGGVSGILQVTSLLILLLLLIKAAQLYLHRQWLLKALQQFPCPPSHWLFGHIQEFQHDQELQRIQERVKTFPSACPYWIWGGKVRVQLYDPDYMKVILGRSDPKSHGSYKFLAPRIGYGLLLLNGQTWFQHRRMLTPAFHNDILKPYVGLMADSVRVMLDKWEELLGQDSPLEVFQHVSLMTLDTIMKSAFSHQGSIQVDRNSQSYIQAISDLNSLVFCCMRNAFHENDTIYSLTSAGRWTHRACQLAHQHTDQVIQLRKAQLQKEGELEKIKRKRHLDFLDILLLAKMENGSILSDKDLRAEVDTFMFEGHDTTASGISWILYALATHPKHQERCREEIHGLLGDGASITWNHLDQMPYTTMCIKEALRLYPPVPGIGRELSTPVTFPDGRSLPKGIMVLLSIYGLHHNPKVWPNLEVFDPSRFAPGSAQHSHAFLPFSGGSRNCIGKQFAMNQLKVARALTLLRFELLPDPTRIPIPMARLVLKSKNGIHLRLRRLPNPCEDKDQL

SEQ ID NO: 10 - protein, 511 aa, Homo sapiens
MVPSFLSLSFSSLGLWASGLILVLGFLKLIHLLLRRQTLAKAMDKFPGPPTHWLFGHALEIQETGSLDKVVSWAHQFPYAHPLWFGQFIGFLNIYEPDYAKAVYSRGDPKAPDVYDFFLQWIGRGLLVLEGPKWLQHRKLLTPGFHYDVLKPYVAVFTESTRIMLDKWEEKAREGKSFDIFCDVGHMALNTLMKCTFGRGDTGLGHRDSSYYLAVSDLTLLMQQRLVSFQYHNDFIYWLTPHGRRFLRACQVAHDHTDQVIRERKAALQDEKVRKKIQNRRHLDFLDILLGARDEDDIKLSDADLRAEVDTFMFEGHDTTTSGISWFLYCMALYPEHQHRCREEVREILGDQDFFQWDDLGKMTYLTMCIKESFRLYPPVPQVYRQLSKPVTFVDGRSLPAGSLISMHIYALHRNSAVWPDPEVFDSLRFSTENASKRHPFAFMPFSAGPRNCIGQQFAMSEMKVVTAMCLLRFEFSLDPSRLPIKMPQLVLRSKNGFHLHLKPLGPGSGK

SEQ ID NO: 11 - protein, 520 aa, Homo sapiens
MSQLSLSWLGLWPVAASPWLLLLLVGASWLLAHVLAWTYAFYDNCRRLRCFPQPPRRNWFWGHQGMVNPTEEGMRVLTQLVATYPQGFKVWMGPISPLLSLCHPDIIRSVINASAAIAPKDKFFYSFLEPWLGDGLLLSAGDKWSRHRRMLTPAFHFNILKPYMKIFNESVNIMHAKWQLLASEGSACLDMFEHISLMTLDSLQKCVFSFDSHCQEKPSEYIAAILELSALVSKRHHEILLHIDFLYYLTPDGQRFRRACRLVHDFTDAVIQERRRTLPSQGVDDFLQAKAKSKTLDFIDVLLLSKDEDGKKLSDEDIRAEADTFMFEGHDTTASGLSWVLYHLAKHPEYQERCRQEVQELLKDREPKEIEWDDLAHLPFLTMCMKESLRLHPPVPVISRHVTQDIVLPDGRVIPKGIICLISVFGTHHNPAVWPDPEVYDPFRFDPENIKERSPLAFIPFSAGPRNCIGQTFAMAEMKVVLALTLLRFRVLPDHTEPRRKPELVLRAEGGLWLRVEPLS

SEQ ID NO: 12 - protein, 520 aa, Homo sapiens
MPQLSLSSLGLWPMAASPWLLLLLVGASWLLARILAWTYTFYDNCCRLRCFPQPPKRNWFLGHLGLIHSSEEGLLYTQSLACTFGDMCCWWVGPWHAIVRIFHPTYIKPVLFAPAAIVPKDKVFYSFLKPWLGDGLLLSAGEKWSRHRRMLTPAFHFNILKPYMKIFNESVNIMHAKWQLLASEGSARLDMFEHISLMTLDSLQKCVFSFDSHCQEKPSEYIAAILELSALVTKRHQQILLYIDFLYYLTPDGQRFRRACRLVHDFTDAVIQERRRTLPSQGVDDFLQAKAKSKTLDFIDVLLLSKDEDGKKLSDEDIRAEADTFMFEGHDTTASGLSWVLYHLAKHPEYQERCRQEVQELLKDREPKEIEWDDLAQLPFLTMCIKESLRLHPPVPAVSRCCTQDIVLPDGRVIPKGIICLISVFGTHHNPAVWPDPEVYDPFRFDPKNIKERSPLAFIPFSAGPRNCIGQAFAMAEMKVVLGLTLLRFRVLPDHTEPRRKPELVLRAEGGLWLRVEPLS

SEQ ID NO: 13 - protein, 520 aa, Homo sapiens
MSLLSLSWLGLRPVAASPWLLLLVVGASWLLARILAWTYAFYHNGRRLRCFPQPRKQNWFLGHLGLVTPTEEGLRVLTQLVATYPQGFVRWLGPITPIINLCHPDIVRSVINTSDAITDKDIVFYKTLKPWLGDGLLLSVGDKWRHHRRLLTPAFHFNILKPYIKIFSKSANIMHAKWQRLAMEGSTCLDVFEHISLMTLDSLQKCIFSFDSNCQEKPSEYITAIMELSALVVKRNNQFFRYKDFLYFLTPCGRRFHRACRLVHDFTDAVIQERRRTLTSQGVDDFLQAKAKSKTLDFIDVLLLSEDKNGKELSDEDIRAEADTFMFGGHDTTASGLSWVLYNLARHPEYQERCRQEVQELLKDREPKEIEWDDLAQLPFLTMCLKESLRLHPPIPTFARGCTQDVVLPDSRVIPKGNVCNINIFAIHHNPSVWPDPEVYDPFRFDPENAQKRSPMAFIPFSAGPRNCIGQKFAMAEMKVVLALTLLRFRILPDHREPRRTPEIVLRAEDGLWLRVEPLG

SEQ ID NO: 14 - protein, 524 aa, Homo sapiens
MPQLSLSWLGLGPVAASPWLLLLLVGGSWLLARVLAWTYTFYDNCRRLQCFPQPPKQNWFWGHQGLVTPTEEGMKTLTQLVTTYPQGFKLWLGPTFPLLILCHPDIIRPITSASAAVAPKDMIFYGFLKPWLGDGLLLSGGDKWSRHRRMLTPAFHFNILKPYMKIFNKSVNIMHDKWQRLASEGSARLDMFEHISLMTLDSLQKCVFSFESNCQEKPSEYIAAILELSAFVEKRNQQILLHTDFLYYLTPDGQRFRRACHLVHDFTDAVIQERRCTLPTQGIDDFLKNKAKSKTLDFIDVLLLSKDEDGKELSDEDIRAEADTFMFEGHDTTASGLSWVLYHLAKHPEYQEQCRQEVQELLKDREPIEIEWDDLAQLPFLTMCIKESLRLHPPVPVISRCCTQDFVLPDGRVIPKGIVCLINIIGIHYNPTVWPDPEVYDPFRFDQENIKERSPLAFIPFSAGPRNCIGQAFAMAEMKVVLALTLLHFRILPTHTEPRRKPELILRAEGGLWLRVEPLGANSQ

SEQ ID NO: 15 - protein, 524 aa, Homo sapiens
MSLLSLPWLGLRPVATSPWLLLLLVVGSWLLARILAWTYAFYNNCRRLQCFPQPPKRNWFWGHLGLITPTEEGLKNSTQMSATYSQGFTVWLGPIIPFIVLCHPDTIRSITNASAAIAPKDNLFIRFLKPWLGEGILLSGGDKWSRHRRMLTPAFHFNILKSYITIFNKSANIMLDKWQHLASEGSSRLDMFEHISLMTLDSLQKCIFSFDSHCQERPSEYIATILELSALVEKRSQHILQHMDFLYYLSHDGRRFHRACRLVHDFTDAVIRERRRTLPTQGIDDFFKDKAKSKTLDFIDVLLLSKDEDGKALSDEDIRAEADTFMFGGHDTTASGLSWVLYNLARHPEYQERCRQEVQELLKDRDPKEIEWDDLAQLPFLTMCVKESLRLHPPAPFISRCCTQDIVLPDGRVIPKGITCLIDIIGVHHNPTVWPDPEVYDPFRFDPENSKGRSPLAFIPFSAGPRNCIGQAFAMAEMKVVLALMLLHFRFLPDHTEPRRKLELIMRAEGGLWLRVEPLNVSLQ

SEQ ID NO: 16 - protein, 531 aa, Homo sapiens
MLPITDRLLHLLGLEKTAFRIYAVSTLLLFLLFFLFRLLLRFLRLCRSFYITCRRLRCFPQPPRRNWLLGHLGMYLPNEAGLQDEKKVLDNMHHVLLVWMGPVLPLLVLVHPDYIKPLLGASAAIAPKDDLFYGFLKPWLGDGLLLSKGDKWSRHRRLLTPAFHFDILKPYMKIFNQSADIMHAKWRHLAEGSAVSLDMFEHISLMTLDSLQKCVFSYNSNCQEKMSDYISAIIELSALSVRRQYRLHHYLDFIYYRSADGRRFRQACDMVHHFTTEVIQERRRALRQQGAEAWLKAKQGKTLDFIDVLLLARDEDGKELSDEDIRAEADTFMFEGHDTTSSGISWMLFNLAKYPEYQEKCREEIQEVMKGRELEELEWDDLTQLPFTTMCIKESLRQYPPVTLVSRQCTEDIKLPDGRIIPKGIICLVSIYGTHHNPTVWPDSKVYNPYRFDPDNPQQRSPLAYVPFSAGPRNCIGQSFAMAELRVVVALTLLRFRLSVDRTRKVRRKPELILRTENGLWLKVEPLPPRA

SEQ ID NO: 17 - protein, 509 aa, Homo sapiens
MEFSWLETRWARPFYLAFVFCLALGLLQAIKLYLRRQRLLRDLRPFPAPPTHWFLGHQKFIQDDNMEKLEEIIEKYPRAFPFWIGPFQAFFCIYDPDYAKTLLSRTDPKSQYLQKFSPPLLGKGLAALDGPKWFQHRRLLTPGFHFNILKAYIEVMAHSVKMMLDKWEKICSTQDTSVEVYEHINSMSLDIIMKCAFSKETNCQTNSTHDPYAKAIFELSKIIFHRLYSLLYHSDIIFKLSPQGYRFQKLSRVLNQYTDTIIQERKKSLQAGVKQDNTPKRKYQDFLDIVLSAKDESGSSFSDIDVHSEVSTFLLAGHDTLAASISWILYCLALNPEHQERCREEVRGILGDGSSITWDQLGEMSYTTMCIKETCRLIPAVPSISRDLSKPLTFPDGCTLPAGITVVLSIWGLHHNPAVWKNPKVFDPLRFSQENSDQRHPYAYLPFSAGSRNCIGQEFAMIELKVTIALILLHFRVTPDPTRPLTFPNHFILKPKNGMYLHLKKLSEC

SEQ ID NO: 18 - protein, 505 aa, Homo sapiens
MEPSWLQELMAHPFLLLILLCMSLLLFQVIRLYQRRRWMIRALHLFPAPPAHWFYGHKEFYPVKEFEVYHKLMEKYPCAVPLWVGPFTMFFSVHDPDYAKILLKRQDPKSAVSHKILESWVGRGLVTLDGSKWKKHRQIVKPGFNISILKIFITMMSESVRMMLNKWEEHIAQNSRLELFQHVSLMTLDSIMKCAFSHQGSIQLDSTLDSYLKAVFNLSKISNQRMNNFLHHNDLVFKFSSQGQIFSKFNQELHQFTEKVIQDRKESLKDKLKQDTTQKRRWDFLDILLSAKSENTKDFSEADLQAEVKTFMFAGHDTTSSAISWILYCLAKYPEHQQRCRDEIRELLGDGSSITWEHLSQMPYTTMCIKECLRLYAPVVNISRLLDKPITFPDGRSLPAGITVFINIWALHHNPYFWEDPQVFNPLRFSRENSEKIHPYAFIPFSAGLRNCIGQHFAIIECKVAVALTLLRFKLAPDHSRPPQPVRQVVLKSKNGIHVFAKKVC

SEQ ID NO: 19 - protein, 525 aa, Pan troglodytes
MAGLWLGLVWQKLLLWGAASAVSLAGASLVLSLLQRVATYARKWQQMRPIPTVARAYPLVGHALLMKPDGREFFQQIIEYTEEYRHMPLLKLWVGPVPMVALYNAENVEVILTSSKQIDKSSMYKFLEPWLGLGLLTSTGNKWRSRRKMLTPTFHFTILEDFLDIMNEQANTLVKKLEKHINQEAFNCFFYITLCALDIICETAMGKNIGAQSNDDSEYVRAVYRMSEMIFRRIKMPWLWLDLWYLMFKEGWEHKKSLKILHTFTNSVIAERANEMNANEDCRGDGRGSAPSKNKRRAFLDLLLSVTDDEGNRLSHEDIREEVDTFMFEGHDTTAAAINWSLYLLGSNPEVQKKVDHELDDVFGKSDRPATVEDLKKLRYLECVIKETLRLFPSVPLFARSVSEDCEVAGYRVLKGTEAVIIPYALHRDPRYFPNPEEFQPERFFPKNAQGRHPYAYVPFSAGPRNCIGQKFAVMEEKTILSCILRHFWIESNQKREELGLEGQLILRPSNGIWIKLKRRNADER

SEQ ID NO: 20 - protein, 525 aa, Macaca mulatta
MAGIWLGLVWQKLLLWGAASAVSLAGASLVLSLLQRVASYVRKWQQMRPIPTVARAYPLVGHALLMKRDGREFFQQIIEYTEEYRHMPLLKLWVGPVPMVALYNAENVEVILTSSKQIDKSSMYKFLEPWLGLGLLTSTGNKWRSRRKMLTPTFHFTILEDFLDIMNEQANILVKKLEKHVNQEAFNCFVYITLCALDIICETAMGKNIGAQSNDDSEYVRAVYRMSEMIFRRIKMPWLWLDLWYLMFKEGWEHKKSLKILHAFTNNVIAERANEMNVDEDCRGDGRDSAPSKNKRRAFLDLLLSVTDDEGNRLSHEDIREEVDTFMFEGHDTTAAAMNWSLYLLGSNPEVQKKVDHELDDVFGRSDRPATVEDLKKLRYLECVIKETLRLFPSVPLFARSVSEDCEVAGYRVLKGTEAVIIPYALHRDPRYFPNPEEFRPERFFPENAQGRHPYAYVPFSAGPRNCIGQKFAVMEEKTILSCILRHFWIESNQKREELGLEGQLILRPTNGIWIKLKRRNADEP

SEQ ID NO: 21 - protein, 539 aa, Canis lupus
MLKVKWKENVFREGDKDSNMLDAVQLPSIKVESALSDAEAGGSPGGRRPVLTVERGRLAQGSMSSLLKNPKDTTRNSLKIKYFLPEFFQQVILYSEESRHLPLLKLWLGPIPIVAIYSAENVEVILTSSRQIDKSYVYKFLEPWLGLGLLTSTGNKWRSRRKMLTPTFHFTILEDFLDVMNEHANILVNKLEKHVNQEAFNCFFYITLCALDIICETAMGKNIGAQNNEDSEYVRAIYRMSDTIHRRMKMPWLWLDFLFLMFKEGREHKRNLEILHNFTNNVITERASELKRDEEHGSADKDCSPSKNKRRAFLDLLLNVTDDEGNKLRHEDVREEVDTFMFEGHDTTAAAINWSLYLLGSYPEVQKQVDSELEDVFGKSDRPATLEDLKKLKYLECVIKESLRLFPSVPLFARNLNEDCVVAGYKVVKGSQAIIIPYALHRDPRYFPNPEEFQPERFFPENLQGRHPYAYIPFSAGPRNCIGQRFAIMEEKTVLSCVLRHFWVESNQKREELGLAGELILRPTNGIWIKLKRRNADES

SEQ ID NO: 22 - protein, 527 aa, Bos Taurus
MLAPWLLSVGPKLLLWSGLCAVSLAGATLTLNLLKMVASYARKWRQMRPVPTIGDPYPLVGHALMMKPDARDFFQQIIDFTEECRHLPLLKLWLGPVPLVALYNAETVEVILSSSKHIEKSYMYKFLEPWLGLGLLTSTGNKWRSRRKMLTPTFHFTILEDFLDVMNEQANILVTKLEKHVNQEAFNCFFYVTLCTLDIICETAMGKNIGAQRNDDSEYVRAVYRMSDSIHQRMKMPWLWLDLIFYMFKNGREHRRSLKIVHDFTNNVITERANEMKRHEEGTSNDKEKDFPPRKTKCRAFLDLLLNVTDDQGNKLSHEDIREEVDTFMFEGHDTTAAAINWSLYLLGWYPEVQQRVDTELEEVFGKSDRPVTLEDLKKLKYLDCVIKESLRLFPSVPFFARNLTEDCEVAGHKIVQGCQVIIVPYALHRDPKYFPDPEEFKPERFFPENLKGRHTYAYVPFSAGPRNCIGQKFAIMEEKTILSCILRHFWVESNQKREELGLAGELILRPSNGIWIKLKRRNTDES

SEQ ID NO: 23 - protein, 525 aa, Mus musculus
MLWLWLGLSGQKLLLWGAASAVSLAGATILISIFPMLVSYARKWQQMRSIPSVARAYPLVGHALYMKPNNAEFFQQLIYYTEEFRHLPIIKLWIGPVPLVALYKAENVEVILTSSKQIDKSFLYKFLQPWLGLGLLTSTGSKWRTRRKMLTPTFHFTILENFLDVMNEQANILVNKLEKHVNQEAFNCFFYITLCALDIICETAMGKNIGAQSNNDSEYVRTVYRMSDMIYRRMKMPWLWFDLWYLVFKEGRDHKRGLKCLHTFTNNVIAERVKERKAEEDWTGAGRGPIPSKNKRKAFLDLLLSVTDEEGNRLSQEDIREEVDTFMFEGHDTTAAAINWSLYLLGTNPEVQRKVDQELDEVFGRSHRPVTLEDLKKLKYLDCVIKETLRVFPSVPLFARSLSEDCEVGGYKVTKGTEAIIIPYALHRDPRYFPDPEEFRPERFFPENSQGRHPYAYVPFSAGPRNCIGQKFAVMEEKTILACILRQFWVESNQKREELGLAGDLILRPNNGIWIKLKRRHEDDP

SEQ ID NO: 24 - protein, 525 aa, Rattus norvegicus
MLWLWLGLSGQKLLLWGAASAVSVAGATVLLNILQMLVSYARKWQQMRPIPSVARAYPLVGHALFMKPNNTEFFQQIIQYTEEFRHLPIIKLWIGPVPLVALYKAENVEVILTSSKQIDKSFMYKFLQPWLGLGLLTSTGSKWRARRKMLTPSFHFTILEDFLDVMNEQANILVNKLEKHVNQEAFNCFFPITLCALDIICETAMGKNIGAQSNGDSEYVRTVYRMSDMIYRRMKMPWFWFDLWYLMFKEGRDHKKGLKSLHTFTNNVIAERVNARKAEQDCIGAGRGPLPSKTKRKAFLDLLLSVTDEEGNKLSHEDIREEVDTFMFEGHDTTAAAINWSLYLLGSNPEVQRKVDKELDDVFGRSHRPVTLEDLKKLKYLDCVIKETLRVFPSVPLFARSLSEDCEVAGYKISKGTEAVIIPYALHRDPRYFPDPEEFQPERFFPENSQGRHPYAYVPFSAGPRNCIGQKFAVMEEKTILACILREFWIESNQKREELGLAGDLILRPNNGIWIKLKRRHEDDP

SEQ ID NO: 25 - protein, 530 aa, Gallus gallus
MAMEITLGSMEGTQLLPWVAGAITLLLTVVTVHFLPSLLNYWWWWWVMKPIPGIRPCYPFVGNALLLERNGEGFFKQLQQYADEFRKMPMFKLWLGPLPVTVLFHPDSVEVILSSSKHIKKSFLYTFLHPWLGTGLLTSTGDKWRSRRKMITPTFHFAILNDFLEVMNEQGGVLLEKLEKHVDKEPFNIFTDITLCALDIICETAMGKNLGAQDNKDSEYVRAVYRMSDLIQQRQKSPWLWHDLMYLLFKEGREHERNLKILHGFTDTVIAEKVAELENTKLTKHDTDVNTEEESGSKKREAFLDMLLNATDDEGKKLSYKDIREEVDTFMFEGHDTTAAAMNWVLYLLGHHPEAQKKVHQELDEVFGNTERPVTVDDLKKLRYLECVVKEALRLFPSVPMFARSLQEDCYISGYKLPKGTNVLVLTYVLHRDPEIFPEPDEFRPERFFPENSKGRHPYAYVPFSAGPRNCIGQRFAQMEEKTLLALILRRFWVDCSQKPEELGLSGELILRPNNGIWVQLKRRPKTVTE

SEQ ID NO: 26 - protein, 523 aa, Xenopus tropicalis
MELGGEVHLLVWVAAAVVLLTLLALSILPALQDYVRKRRILKPIPGPGPNYPLIGDALFLKNNGGDFFLQICEYTESYRLQPLLKVWIGTIPFIVVYHADTVEPVLSSSKHMDKAFLYKFLHPWLGKGLLTSTGEKWRSRRKMITPTFHFAILSEFLEVMNEQSKILVEKLQTHVDGESFDCFMDVTLCALDIISETAMGRKIQAQSNRDSEYVQAIYKMSDIIQRRQKMPWLWLDFLYAHLRDGKEHDKNLKILHSFTDKAILERAEELKKMGEQKKEHCDSDPESDKPKKRSAFLDMLLMATDDAGNKMSYMDIREEVDTFMFEGHDTTAAALNWSLFLLGSHPEAQRQVHKELDEVFGKSDRPVTMDDLKKLRYLEAVIKESLRIYPSVPLFGRTVTEDCSIRGFHVPKGVNVVIIPYALHRDPEYFPEPEEFRPERFFPENASGRNPYAYIPFSAGLRNCIGQRFALMEEKVVLSSILRNYWVEASQKREELCLLGELILRPQDGMWIKLKNRETAPTA

SEQ ID NO: 27 - protein, 469 aa, Equus caballus
MFVLIEFKIKYSLSDFFQQLIYYTEENRHLPLLKLWLGPVPVVIFYNAENVEVILTSSRQIDKSYMYKFLKPWLGLGLLTSTGNKWRSRRKMLTPTFHFTNLEDFLDVMNEQANILVNKLEKHVNQEAFNCFLYITLCALDIICETAMGKNIGAQRNNDSEYVRAVYRMSDMIHRRMKMPWLWLDIFFLMFKEGREHRRLLKILHNFTNNVIVERASEMKKDEERSRSDDGGSAPSKNKRRAFLDLLLNVTDDEGNKLSHEDIRQEVDTFMFEGHDTTAAAINWSLYLLGCYPEVQKKVDSELEEVFGKSDRPATLEDLKKLKYLECVMKETLRLFPSVPLFARNLNEDCEVAGYKIVKGSQAIIVSYALHRDSRYFPNPEEFKPERFFPENSQGRHPYAYVPFSAGPRNCIGQKFAVMEEKIILSCILRHFWVESNQKREELGLAGELILRPSNGIWIKLKRRNTEES

SEQ ID NO: 28 - protein, 524 aa, Oryctolagus cuniculus
MWLWLGLVGQKLLFWGAASAVSLAGASLFLNLLQMVASYARKWQQMRPIPTIGRPYPLVGHALYMKPSGKEFFQQLIQYTEEYRHLPLLKLWLGPLPIVALYNAENVEVILNSSKQINKSSMYQFLEPWLGLGLLTSTGYKWRSRRKMLTPTFHFTILEDFLDIMNEQANILVHKLEKHVDQEAFNCFFYITLCALDIICETAMGKNIGAQSNEDSEYVRAVYRMSDVIFRRMKMPWLWLDLWYLMFKEGWEHKRCLKILHRFTNNVIAERVSEMKTDEEHRDADSNCAPSTMKRKAFLDLLLTVTDEEGNKLSHEDIREEVDTFMFEGHDTTAAAINWSLYLLGSHPEVQRKVDDELDEVFGKSDRPATSEDLKKLKYLECVIKETLRLFPSVPLFARSLSDDCEVAGFRVVKGTQAVIVPYALHRDPKYFPNPEEFRPERFFPENAQGRHPYAYVPFSAGPRNCIGQKFAIMEEKTILSCILRKLWVESNQKMEELGLAGELILRPTNGIWIKLKRRNADKA

SEQ ID NO: 29 - protein, 535 aa, Drosophila melanogaster
MSSKVITSLMAESILLSKVGQVISGYSPITVFLLGSILIFLVVYNKRRSRLVKYIEKIPGPAAMPFLGNAIEMNVDHDELFNRVIGMQKLWGTRIGINRVWQGTAPRVLLFEPETVEPILNSQKFVNKSHDYDYLHPWLGEGLLTSTDRKWHSRRKILTPAFHFKILDDFIDVFNEQSAVLARKLAVEVGSEAFNLFPYVTLCTLDIVCETAMGRRIYAQSNSESEYVKAVYGIGSIVQSRQAKIWLQSDFIFSLTAEYKLHQSYINTLHGFSNMVIRERKAELAILQENNNNNNNNAPDAYDDVGKKKRLAFLDLLIDASKEGTVLSNEDIREEVDTFMFEGHDTTSAAISWTLFLLGCHPEYQERVVEELDSIFGDDKETPATMKNLMDMRYLECCIKDSLRLFPSVPMMARMVGEDVNIGGKIVPAGTQAIIMTYALHRNPRVFPKPEQFNPDNFLPENCAGRHPFAYIPFSAGPRNCIGQKFAILEEKAVISTVLRKYKIEAVDRREDLTLLGELILRPKDGLRVKITPRD

SEQ ID NO: 30 - protein, 10 aa, synthetic construct
  REGION 1..10: note = Synthetically generated consensus sequence
  REGION 2..3: note = misc_feature - Xaa can be any naturally occurring amino acid
  REGION 5..7: note = misc_feature - Xaa can be any naturally occurring amino acid
  SITE 9: note = misc_feature - Xaa can be any naturally occurring amino acid
FXXGXXXCXG

SEQ ID NO: 31 - skipped

SEQ ID NO: 32 - DNA, 1715 bp, synthetic construct
  misc_feature 1..1715: note = Synthetically generated promoter sequence
  source 1..1715: mol_type = other DNA
gacattgattattgactagttattaatagtaatcaattacggggtcattagttcatagcccatatatggagttccgcgttacataacttacggtaaatggcccgcctggctgaccgcccaacgacccccgcccattgacgtcaataatgacgtatgttcccatagtaacgccaatagggactttccattgacgtcaatgggtggactatttacggtaaactgcccacttggcagtacatcaagtgtatcatatgccaagtacgccccctattgacgtcaatgacggtaaatggcccgcctggcattatgcccagtacatgaccttatgggactttcctacttggcagtacatctacgtattagtcatcgctattaccatgggtcgaggtgagccccacgttctgcttcactctccccatctcccccccctccccacccccaattttgtatttatttattttttaattattttgtgcagcgatgggggcggggggggggggggcgcgcgccaggcggggcggggcggggcgaggggcggggcggggcgaggcggagaggtgcggcggcagccaatcagagcggcgcgctccgaaagtttccttttatggcgaggcggcggcggcggcggccctataaaaagcgaagcgcgcggcgggcgggagtcgctgcgttgccttcgccccgtgccccgctccgcgccgcctcgcgccgcccgccccggctctgactgaccgcgttactcccacaggtgagcgggcgggacggcccttctcctccgggctgtaattagcgcttggtttaatgacggctcgtttcttttctgtggctgcgtgaaagccttaaagggctccgggagggccctttgtgcgggggggagcggctcggggggtgcgtgcgtgtgtgtgtgcgtggggagcgccgcgtgcggcccgcgctgcccggcggctgtgagcgctgcgggcgcggcgcggggctttgtgcgctccgcgtgtgcgcgaggggagcgcggccgggggcggtgccccgcggtgcgggggggctgcgaggggaacaaaggctgcgtgcggggtgtgtgcgtgggggggtgagcagggggtgtgggcgcggcggtcgggctgtaacccccccctgcacccccctccccgagttgctgagcacggcccggcttcgggtgcggggctccgtgcggggcgtggcgcggggctcgccgtgccgggcggggggtggcggcaggtgggggtgccgggcggggcggggccgcctcgggccggggagggctcgggggaggggcgcggcggccccggagcgccggcggctgtcgaggcgcggcgagccgcagccattgccttttatggtaatcgtgcgagagggcgcagggacttcctttgtcccaaatctggcggagccgaaatctgggaggcgccgccgcaccccctctagcgggcgcgggcgaagcggtgcggcgccggcaggaaggaaatgggcggggagggccttcgtgcgtcgccgcgccgccgtccccttctccatctccagcctcggggctgccgcagggggacggctgccttcgggggggacggggcagggcggggttcggcttctggcgtgtgaccggcggctctagagcctctgctaaccatgttcatgccttcttctttttcctacagctcctgggcaacgtgctggttattgtgctgtctcatcattttggcaaa

SEQ ID NO: 33 - DNA, 589 bp, Woodchuck hepatitis virus
  source 1..589: mol_type = unassigned DNA
aatcaacctctggattacaaaatttgtgaaagattgactggtattcttaactatgttgctccttttacgctatgtggatacgctgctttaatgcctttgtatcatgctattgcttcccgtatggctttcattttctcctccttgtataaatcctggttgctgtctctttatgaggagttgtggcccgttgtcaggcaacgtggcgtggtgtgcactgtgtttgctgacgcaacccccactggttggggcattgccaccacctgtcagctcctttccgggactttcgctttccccctccctattgccacggcggaactcatcgccgcctgccttgcccgctgctggacaggggctcggctgttgggcactgacaattccgtggtgttgtcggggaaatcatcgtcctttccttggctgctcgcctgtgttgccacctggattctgcgcgggacgtccttctgctacgtcccttcggccctcaatccagcggaccttccttcccgcggcctgctgccggctctgcggcctcttccgcgtcttcgccttcgccctcagacgagtcggatctccctttgggccgcctccccgc

SEQ ID NO: 34 - DNA, 225 bp, Bos Taurus
  source 1..225: mol_type = unassigned DNA
ctgtgccttctagttgccagccatctgttgtttgcccctcccccgtgccttccttgaccctggaaggtgccactcccactgtcctttcctaataaaatgaggaaattgcatcgcattgtctgagtaggtgtcattctattctggggggtggggtggggcaggacagcaagggggaggattgggaagacaatagcaggcatgctggggatgcggtgggctctatgg

SEQ ID NO: 35 - DNA, 235 bp, synthetic construct
  misc_feature 1..235: note = Synthetically generated promoter sequence
  source 1..235: mol_type = other DNA
gattggctccggtgcccgtcagtgggcagagcgcacatcgcccacagtccccgagaagttggggggaggggtcggcaattgaaccggtgcctagagaaggtggcgcggggtaaactgggaaagtgatgtcgtgtactggctccgcctttttcccgagggtgggggagaaccgtatataagtgcagtagtcgccgtgaacgttctttttcgcaacgggtttgccgccagaacacag

SEQ ID NO: 36 - DNA, 54 bp, synthetic construct
  misc_feature 1..54: note = Synthetically generated signal sequence
  source 1..54: mol_type = other DNA
gatccaataaaagatctttattttcattagatctgtgtgttggttttttgtgtg

SEQ ID NO: 37-38 - skipped (2 entries)

SEQ ID NO: 39 - DNA, 120 bp, Simian virus 40
  source 1..120: mol_type = unassigned DNA
ttgtttattgcagcttataatggttacaaataaagcaatagcatcacaaatttcacaaataaagcatttttttcactgcattctagttgtggtttgtccaaactcatcaatgtatcttat

SEQ ID NO: 40 - DNA, 576 bp, Cytomegalovirus
  source 1..576: mol_type = unassigned DNA
tagtaatcaattacggggtcattagttcatagcccatatatggagttccgcgttacataacttacggtaaatggcccgcctggctgaccgcccaacgacccccgcccattgacgtcaataatgacgtatgttcccatagtaacgccaatagggactttccattgacgtcaatgggtggagtatttacggtaaactgcccacttggcagtacatcaagtgtatcatatgccaagtacgccccctattgacgtcaatgacggtaaatggcccgcctggcattatgcccagtacatgaccttatgggactttcctacttggcagtacatctacgtattagtcatcgctattaccatggtgatgcggttttggcagtacatcaatgggcgtggatagcggtttgactcacggggatttccaagtctccaccccattgacgtcaatgggagtttgttttggcaccaaaatcaacgggactttccaaaatgtcgtaacaactccgccccattgacgcaaatgggcggtaggcgtgtacggtgggaggtctatataagcagagctggtttagtgaaccgtcag

SEQ ID NO: 41 - DNA, 1184 bp, Homo sapiens
  source 1..1184: mol_type = unassigned DNA
cgtgaggctccggtgcccgtcagtgggcagagcgcacatcgcccacagtccccgagaagttggggggaggggtcggcaattgaaccggtgcctagagaaggtggcgcggggtaaactgggaaagtgatgtcgtgtactggctccgcctttttcccgagggtgggggagaaccgtatataagtgcagtagtcgccgtgaacgttctttttcgcaacgggtttgccgccagaacacaggtaagtgccgtgtgtggttcccgcgggcctggcctctttacgggttatggcccttgcgtgccttgaattacttccacctggctgcagtacgtgattcttgatcccgagcttcgggttggaagtgggtgggagagttcgaggccttgcgcttaaggagccccttcgcctcgtgcttgagttgaggcctggcctgggcgctggggccgccgcgtgcgaatctggtggcaccttcgcgcctgtctcgctgctttcgataagtctctagccatttaaaatttttgatgacctgctgcgacgctttttttctggcaagatagtcttgtaaatgcgggccaagatctgcacactggtatttcggtttttggggccgcgggcggcgacggggcccgtgcgtcccagcgcacatgttcggcgaggcggggcctgcgagcgcggccaccgagaatcggacgggggtagtctcaagctggccggcctgctctggtgcctggcctcgcgccgccgtgtatcgccccgccctgggcggcaaggctggcccggtcggcaccagttgcgtgagcggaaagatggccgcttcccggccctgctgcagggagctcaaaatggaggacgcggcgctcgggagagcgggcgggtgagtcacccacacaaaggaaaagggcctttccgtcctcagccgtcgcttcatgtgactccacggagtaccgggcgccgtccaggcacctcgattagttctcgagcttttggagtacgtcgtctttaggttggggggaggggttttatgcgatggagtttccccacactgagtgggtggagactgaagttaggccagcttggcacttgatgtaattctccttggaatttgccctttttgagtttggatcttggttcattctcaagcctcagacagtggttcaaagtttttttcttccatttcaggtgtcgtga

SEQ ID NO: 42 - DNA, 141 bp, Adeno-associated virus
  source 1..141: mol_type = unassigned DNA
cctgcaggcagctgcgcgctcgctcgctcactgaggccgcccgggcaaagcccgggcgtcgggcgacctttggtcgcccggcctcagtgagcgagcgagcgcgcagagagggagtggccaactccatcactaggggttcct

SEQ ID NO: 43 - DNA, 141 bp, Adeno-associated virus
  source 1..141: mol_type = unassigned DNA
aggaacccctagtgatggagttggccactccctctctgcgcgctcgctcgctcactgaggccgggcgaccaaaggtcgcccgacgcccgggctttgcccgggcggcctcagtgagcgagcgagcgcgcagctgcctgcagg

SEQ ID NO: 44 - DNA, 117 bp, synthetic construct
  misc_feature 1..117: note = Synthetically generated mutant adeno-associated virus 2 inverted terminal repeat sequence
  source 1..117: mol_type = other DNA
cctgcaggcagctgcgcgctcgctcgctcactgaggccgcccgggcaaagcccgggcgtcgggcgacctttggtcgcccggcctcagtgagcgagcgagcgcgcagagagggagtgg

SEQ ID NO: 45 - DNA, 141 bp, Adeno-associated virus; identical to SEQ ID NO: 43
  source 1..141: mol_type = unassigned DNA

SEQ ID NO: 46 - DNA, 60 bp, Homo sapiens
  source 1..60: mol_type = unassigned DNA
caaacagaagcatgtgattatcattcaaagcgaacgggccaatgaaatgaacgccaatga

SEQ ID NO: 47 - DNA, 75 bp, Homo sapiens
  source 1..75: mol_type = unassigned DNA
caaacagaagcatgtgattatcattcaaatcatacaggtcatcgctgaacgggccaatgaaatgaacgccaatga

SEQ ID NO: 48 - RNA, 20 nt, synthetic construct
  misc_feature 1..20: note = Synthetically generated oligonucleotide
  source 1..20: mol_type = other RNA
tgattatcattcaaagcgaa

SEQ ID NO: 49 - RNA, 20 nt, synthetic construct
  misc_feature 1..20: note = Synthetically generated oligonucleotide
  source 1..20: mol_type = other RNA
gattatcattcaaagcgaac

SEQ ID NO: 50 - RNA, 20 nt, synthetic construct
  misc_feature 1..20: note = Synthetically generated oligonucleotide
  source 1..20: mol_type = other RNA
gataatcacatgcttctgtt

SEQ ID NO: 51 - RNA, 20 nt, synthetic construct
  misc_feature 1..20: note = Synthetically generated oligonucleotide
  source 1..20: mol_type = other RNA
ttcattggcgttcatttcat

SEQ ID NO: 52 - RNA, 20 nt, synthetic construct
  misc_feature 1..20: note = Synthetically generated oligonucleotide
  source 1..20: mol_type = other RNA
cacatgcttctgtttggact

SEQ ID NO: 53 - RNA, 16 nt, synthetic construct
  misc_feature 1..16: note = Synthetically generated oligonucleotide
  source 1..16: mol_type = other RNA
gttttagagctatgct

SEQ ID NO: 54 - RNA, 67 nt, synthetic construct
  misc_feature 1..67: note = Synthetically generated oligonucleotide
  source 1..67: mol_type = other RNA
agcatagcaagttaaaataaggctagtccgttatcaacttgaaaaagtggcaccgagtcggtgcttt

SEQ ID NO: 55 - DNA, 82 bp, synthetic construct
  misc_feature 1..82: note = Synthetically generated oligonucleotide
  source 1..82: mol_type = other DNA
gttttagagctagaaatagcaagttaaaataaggctagtccgttatcaacttgaaaaagtggcaccgagtcggtgctttttt

SEQ ID NO: 56 - DNA, 200 bp, synthetic construct
  misc_feature 1..200: note = Synthetically generated oligonucleotide
  source 1..200: mol_type = other DNA
agaaaaataaatgaaagaaactagcatattttataagaaaatgtgttaactagggtgcatccaagtccaaacagaagcatgtgattatcattcaaatcatacaggtcatcgctgaacgggccaatgaaatgaacgccaatgaagactgtagaggtgatggcaggggctctgccccctccaaaaataaacgcagggccttt

SEQ ID NO: 57 - DNA, 200 bp, synthetic construct
  misc_feature 1..200: note = Synthetically generated oligonucleotide
  source 1..200: mol_type = other DNA
aaaggccctgcgtttatttttggagggggcagagcccctgccatcacctctacagtcttcattggcgttcatttcattggcccgttcagcgatgacctgtatgatttgaatgataatcacatgcttctgtttggacttggatgcaccctagttaacacattttcttataaaatatgctagtttctttcatttatttttct

SEQ ID NO: 58 - protein, 1368 aa, Streptococcus pyogenes [sequence omitted]

SEQ ID NO: 59 - skipped

SEQ ID NO: 60 - DNA, 4799 bp, synthetic construct
  misc_feature 1..4799: note = Synthetically generated expression construct
  source 1..4799: mol_type = other DNA
cctgcaggcagctgcgcgctcgctcgctcactgaggccgcccgggcaaagcccgggcgtcgggcgacctttggtcgcccggcctcagtgagcgagcgagcgcgcagagagggagtggccaactccatcactaggggttcctgcggccaattcagtcgataactataacggtcctaaggtagcgatttaaatacgcgctctcttaaggtagccccgggacgcgtcaattgagatctcgacattgattattgactagttattaatagtaatcaattacggggtcattagttcatagcccatatatggagttccgcgttacataacttacggtaaatggcccgcctggctgaccgcccaacgacccccgcccattgacgtcaataatgacgtatgttcccatagtaacgccaatagggactttccattgacgtcaatgggtggactatttacggtaaactgcccacttggcagtacatcaagtgtatcatatgccaagtacgccccctattgacgtcaatgacggtaaatggcccgcctggcattatgcccagtacatgaccttatgggactttcctacttggcagtacatctacgtattagtcatcgctattaccatgggtcgaggtgagccccacgttctgcttcactctccccatctcccccccctccccacccccaattttgtatttatttattttttaattattttgtgcagcgatgggggcggggggggggggggcgcgcgccaggcggggcggggcggggcgaggggcggggcggggcgaggcggagaggtgcggcggcagccaatcagagcggcgcgctccgaaagtttccttttatggcgaggcggcggcggcggcggccctataaaaagcgaagcgcgcggcgggcgggagtcgctgcgttgccttcgccccgtgccccgctccgcgccgcctcgcgccgcccgccccggctctgactgaccgcgttactcccacaggtgagcgggcgggacggcccttctcctccgggctgtaattagcgcttggtttaatgacggctcgtttcttttctgtggctgcgtgaaagccttaaagggctccgggagggccctttgtgcgggggggagcggctcggggggtgcgtgcgtgtgtgtgtgcgtggggagcgccgcgtgcggcccgcgctgcccggcggctgtgagcgctgcgggcgcggcgcggggctttgtgcgctccgcgtgtgcgcgaggggagcgcggccgggggcggtgccccgcggtgcgggggggctgcgaggggaacaaaggctgcgtgcggggtgtgtgcgtgggggggtgagcagggggtgtgggcgcggcggtcgggctgtaacccccccctgcacccccctccccgagttgctgagcacggcccggcttcgggtgcggggctccgtgcggggcgtggcgcggggctcgccgtgccgggcggggggtggcggcaggtgggggtgccgggcggggcggggccgcctcgggccggggagggctcgggggaggggcgcggcggccccggagcgccggcggctgtcgaggcgcggcgagccgcagccattgccttttatggtaatcgtgcgagagggcgcagggacttcctttgtcccaaatctggcggagccgaaatctgggaggcgccgccgcaccccctctagcgggcgcgggcgaagcggtgcggcgccggcaggaaggaaatgggcggggagggccttcgtgcgtcgccgcgccgccgtccccttctccatctccagcctcggggctgccgcagggggacggctgccttcgggggggacggggcagggcggggttcggcttctggcgtgtgaccggcggctctagagcctctgctaaccatgttcatgccttcttctttttcctacagctcctgggcaacgtgctggttattgtgctgtctcatcattttggcaaagaattctaatacgactcactatagggagacccaagctggctagagccaccatggctggactgtggctgggactggtgtggcagaaactgctgctgtggggggccgcttccgcactgtcactggctggggcttcactggtgctgagcctgctgcagagggtggcctcctacgccagaaagtggcagcagatgaggcccatccctaccgtggccagagcctatccactggtgggacacgcactgctgatgaagcctgacggcagagagttctttcagcagatcatcgagtacacagaggagtataggcacatgccactgctgaagctgtgggtgggacccgtgcctatggtggccctgtacaacgccgagaatgtggaagtgatcctgaccagcagcaagcagatcgataagtctagcatgtataagttcctggagccttggctgggcctgggcctgctgacctctacaggcaacaagtggaggagccggagaaagatgctgaccccaacattccactttacaatcctggaggacttcctggacatcatgaacgagcaggccaatatcctggtgaagaagctggagaagcacatcaaccaggaggcctttaattgcttcttttacatcaccctgtgcgccctggacatcatctgtgagacagctatgggcaagaacatcggcgcccagtctaatgacgatagcgagtacgtgcgggccgtgtatagaatgagcgagatgatctttaggcgcatcaagatgccctggctgtggctggatctgtggtatctgatgttcaaggagggctgggagcacaagaagtccctgcagatcctgcacacctttacaaactctgtgatcgccgagagagccaatgagatgaacgccaatgaggactgtaggggcgatggaaggggcagcgccccttccaagaacaagcggagagccttcctggacctgctgctgagcgtgaccgacgatgagggcaatcgcctgtcccacgaggacatccgggaggaggtggatacattcatgtttgagggacacgacaccacagccgccgccatcaactggtccctgtacctgctgggctctaatccagaggtgcagaagaaggtggatcacgagctggacgacgtgttcggcaagtccgacaggccagcaaccgtggaggatctgaagaagctgagatacctggagtgcgtgatcaaggagacactgcgcctgttcccctctgtgcctctgtttgcccggtccgtgtctgaggactgtgaggtggccggctatcgcgtgctgaagggcaccgaggccgtgatcatcccttacgccctgcaccgggaccccaggtatttccctaacccagaggagtttcagccagagagattctttcccgagaatgcccagggcaggcacccttacgcctatgtgccattctccgccggaccaaggaactgcatcggacagaagtttgccgtgatggaggagaaaaccatcctgtcttgtatcctgagacacttctggatcgagagcaatcagaagagggaggagctgggcctggagggacagctgatcctgcggccaagcaacggcatctggatcaaactgaaaagaaggaacgctgacgagaggtaaaagcttggtaccgatatcgcggccgccctagggagctcctcgaggcggcccgctcgagtctagagggcccttcgaaggtaagcctatccctaaccctctcctcggtctcgattctacgcgtaccggtcatcatcaccatcaccattgagtttcgataatcaacctctggattacaaaatttgtgaaagattgactggtattcttaactatgttgctccttttacgctatgtggatacgctgctttaatgcctttgtatcatgctattgcttcccgtatggctttcattttctcctccttgtataaatcctggttgctgtctctttatgaggagttgtggcccgttgtcaggcaacgtggcgtggtgtgcactgtgtttgctgacgcaacccccactggttggggcattgccaccacctgtcagctcctttccgggactttcgctttccccctccctattgccacggcggaactcatcgccgcctgccttgcccgctgctggacaggggctcggctgttgggcactgacaattccgtggtgttgtcggggaaatcatcgtcctttccttggctgctcgcctgtgttgccacctggattctgcgcgggacgtccttctgctacgtcccttcggccctcaatccagcggaccttccttcccgcggcctgctgccggctctgcggcctcttccgcgtcttcgccttcgccctcagacgagtcggatctccctttgggccgcctccccgcatcgaaacccgctgatcagcctcgactgtgccttctagttgccagccatctgttgtttgcccctcccccgtgccttccttgaccctggaaggtgccactcccactgtcctttcctaataaaatgaggaaattgcatcgcattgtctgagtaggtgtcattctattctggggggtggggtggggcaggacagcaagggggaggattgggaagacaatagcaggcatgctggggatgcggtgggctctatggcttctgaggcggaaagaaccagatcctctcttaaggtagcatcgagatttaaattagggataacagggtaatggcgcgggccgcaggaacccctagtgatggagttggccactccctctctgcgcgctcgctcgctcactgaggccgggcgaccaaaggtcgcccgacgcccgggctttgcccgggcggcctcagtgagcgagcgagcgcgcagctgcctgcagg

SEQ ID NO: 61 - DNA, 4539 bp, synthetic construct
  misc_feature 1..4539: note = Synthetically generated expression construct
  source 1..4539: mol_type = other DNA
cctgcaggcagctgcgcgctcgctcgctcactgaggccgcccgggcaaagcccgggcgtcgggcgacctttggtcgcccggcctcagtgagcgagcgagcgcgcagagagggagtggccaactccatcactaggggttcctgcggcctaaggcaattgagatctcgacattgattattgactagttattaatagtaatcaattacggggtcattagttcatagcccatatatggagttccgcgttacataacttacggtaaatggcccgcctggctgaccgcccaacgacccccgcccattgacgtcaataatgacgtatgttcccatagtaacgccaatagggactttccattgacgtcaatgggtggactatttacggtaaactgcccacttggcagtacatcaagtgtatcatatgccaagtacgccccctattgacgtcaatgacggtaaatggcccgcctggcattatgcccagtacatgaccttatgggactttcctacttggcagtacatctacgtattagtcatcgctattaccatgggtcgaggtgagccccacgttctgcttcactctccccatctcccccccctccccacccccaattttgtatttatttattttttaattattttgtgcagcgatgggggcggggggggggggggcgcgcgccaggcggggcggggcggggcgaggggcggggcggggcgaggcggagaggtgcggcggcagccaatcagagcggcgcgctccgaaagtttccttttatggcgaggcggcggcggcggcggccctataaaaagcgaagcgcgcggcgggcgggagtcgctgcgttgccttcgccccgtgccccgctccgcgccgcctcgcgccgcccgccccggctctgactgaccgcgttactcccacaggtgagcgggcgggacggcccttctcctccgggctgtaattagcgcttggtttaatgacggctcgtttcttttctgtggctgcgtgaaagccttaaagggctccgggagggccctttgtgcgggggggagcggctcggggggtgcgtgcgtgtgtgtgtgcgtggggagcgccgcgtgcggcccgcgctgcccggcggctgtgagcgctgcgggcgcggcgcggggctttgtgcgctccgcgtgtgcgcgaggggagcgcggccgggggcggtgccccgcggtgcgggggggctgcgaggggaacaaaggctgcgtgcggggtgtgtgcgtgggggggtgagcagggggtgtgggcgcggcggtcgggctgtaacccccccctgcacccccctccccgagttgctgagcacggcccggcttcgggtgcggggctccgtgcggggcgtggcgcggggctcgccgtgccgggcggggggtggcggcaggtgggggtgccgggcggggcggggccgcctcgggccggggagggctcgggggaggggcgcggcggccccggagcgccggcggctgtcgaggcgcggcgagccgcagccattgccttttatggtaatcgtgcgagagggcgcagggacttcctttgtcccaaatctggcggagccgaaatctgggaggcgccgccgcaccccctctagcgggcgcgggcgaagcggtgcggcgccggcaggaaggaaatgggcggggagggccttcgtgcgtcgccgcgccgccgtccccttctccatctccagcctcggggctgccgcagggggacggctgccttcgggggggacggggcagggcggggttcggcttctggcgtgtgaccggcggctctagagcctctgctaaccatgttcatgccttcttctttttcctacagctcctgggcaacgtgctggttattgtgctgtctcatcattttggcaaagaattctaatacgactcactatagggagacccaagctggctagccaaagcttccaccatggcggggctctggctggggctcgtgtggcagaagctgctgctgtggggcgcggcgagtgccctttccctggccggcgccagtctggtcctgagcctgctgcagagggtggcgagctacgcgcggaaatggcagcagatgcggcccatccccacggtggcccgcgcctacccactggtgggccacgcgctgctgatgaagccggacgggcgagaattttttcagcagatcattgagtacacagaggaataccgccacatgccgctgctgaagctctgggtcgggccagtgcccatggtggccctttataatgcagaaaatgtggaggtaattttaactagttcaaagcaaattgacaaatcctctatgtacaagtttttagaaccatggcttggcctaggacttcttacaagtactggaaacaaatggcgctccaggagaaagatgttaacacccactttccattttaccattctggaagatttcttagatatcatgaatgaacaagcaaatatattggttaagaaacttgaaaaacacattaaccaagaagcatttaactgctttttttacatcactctttgtgccttagatatcatctgtgaaacagctatggggaagaatattggtgctcaaagtaatgatgattccgagtatgtccgtgcagtttatagaatgagtgagatgatatttcgaagaataaagatgccctggctttggcttgatctctggtaccttatgtttaaagaaggatgggaacacaaaaagagccttcagatcctacatacttttaccaacagtgtcatcgctgaacgggccaatgaaatgaacgccaatgaagactgtagaggtgatggcaggggctctgccccctccaaaaataaacgcagggcctttcttgacttgcttttaagtgtgactgatgacgaagggaacaggctaagtcatgaagatattcgagaagaagttgacaccttcatgtttgaggggcacgatacaactgcagctgcaataaactggtccttatacctgttgggttctaacccagaagtccagaaaaaagtggatcatgaattggatgacgtgtttgggaagtctgaccgtcccgctacagtagaagacctgaagaaacttcggtatctggaatgtgttattaaggagacccttcgcctttttccttctgttcctttatttgcccgtagtgttagtgaagattgtgaagtggcaggttacagagttctaaaaggcactgaagccgtcatcattccctatgcattgcacagagatccgagatacttccccaaccccgaggagttccagcctgagcggttcttccccgagaatgcacaagggcgccatccatatgcctacgtgcccttctctgctggccccaggaactgtataggtcaaaagtttgctgtgatggaagaaaagaccattctttcgtgcatcctgaggcacttttggatagaatccaaccagaaaagagaagagcttggtctagaaggacagttgattcttcgtccaagtaatggcatctggatcaagttgaagaggagaaatgcagatgaacgctaagcggccgcaactcgagactctagaggttaatcgataatcaacctctggattacaaaatttgtgaaagattgactggtattcttaactatgttgctccttttacgctatgtggatacgctgctttaatgcctttgtatcatgctattgcttcccgtatggctttcattttctcctccttgtataaatcctggttgctgtctctttatgaggagttgtggcccgttgtcaggcaacgtggcgtggtgtgcactgtgtttgctgacgcaacccccactggttggggcattgccaccacctgtcagctcctttccgggactttcgctttccccctccctattgccacggcggaactcatcgccgcctgccttgcccgctgctggacaggggctcggctgttgggcactgacaattccgtggtgttgtcggggaaatcatcgtcctttccttggctgctcgcctgtgttgccacctggattctgcgcgggacgtccttctgctacgtcccttcggccctcaatccagcggaccttccttcccgcggcctgctgccggctctgcggcctcttccgcgtcttcgccttcgccctcagacgagtcggatctccctttgggccgcctccccgcatcgaaacccgctgactagacgactgtgccttctagttgccagccatctgttgtttgcccctcccccgtgccttccttgaccctggaaggtgccactcccactgtcctttcctaataaaatgaggaaattgcatcgcattgtctgagtaggtgtcattctattctggggggtggggtggggcaggacagcaagggggaggattgggaagacaatagcaggcatgctggggatgcggtgggctctatggccgcgggccgcaggaacccctagtgatggagttggccactccctctctgcgcgctcgctcgctcactgaggccgggcgaccaaaggtcgcccgacgcccgggctttgcccgggcggcctcagtgagcgagcgagcgcgcagctgcctgcagg

SEQ ID NO: 62 - DNA, 4539 bp, synthetic construct
  misc_feature 1..4539: note = Synthetically generated expression construct
  source 1..4539: mol_type = other DNA
cctgcaggcagctgcgcgctcgctcgctcactgaggccgcccgggcaaagcccgggcgtcgggcgacctttggtcgcccggcctcagtgagcgagcgagcgcgcagagagggagtggccaactccatcactaggggttcctgcggcctaaggcaattgagatctcgacattgattattgactagttattaatagtaatcaattacggggtcattagttcatagcccatatatggagttccgcgttacataacttacggtaaatggcccgcctggctgaccgcccaacgacccccgcccattgacgtcaataatgacgtatgttcccatagtaacgccaatagggactttccattgacgtcaatgggtggactatttacggtaaactgcccacttggcagtacatcaagtgtatcatatgccaagtacgccccctattgacgtcaatgacggtaaatggcccgcctggcattatgcccagtacatgaccttatgggactttcctacttggcagtacatctacgtattagtcatcgctattaccatgggtcgaggtgagccccacgttctgcttcactctccccatctcccccccctccccacccccaattttgtatttatttattttttaattattttgtgcagcgatgggggcggggggggggggggcgcgcgccaggcggggcggggcggggcgaggggcggggcggggcgaggcggagaggtgcggcggcagccaatcagagcggcgcgctccgaaagtttccttttatggcgaggcggcggcggcggcggccctataaaaagcgaagcgcgcggcgggcgggagtcgctgcgttgccttcgccccgtgccccgctccgcgccgcctcgcgccgcccgccccggctctgactgaccgcgttactcccacaggtgagcgggcgggacggcccttctcctccgggctgtaattagcgcttggtttaatgacggctcgtttcttttctgtggctgcgtgaaagccttaaagggctccgggagggccctttgtgcgggggggagcggctcggggggtgcgtgcgtgtgtgtgtgcgtggggagcgccgcgtgcggcccgcgctgcccggcggctgtgagcgctgcgggcgcggcgcggggctttgtgcgctccgcgtgtgcgcgaggggagcgcggccgggggcggtgccccgcggtgcgggggggctgcgaggggaacaaaggctgcgtgcggggtgtgtgcgtgggggggtgagcagggggtgtgggcgcggcggtcgggctgtaacccccccctgcacccccctccccgagttgctgagcacggcccggcttcgggtgcggggctccgtgcggggcgtggcgcggggctcgccgtgccgggcggggggtggcggcaggtgggggtgccgggcggggcggggccgcctcgggccggggagggctcgggggaggggcgcggcggccccggagcgccggcggctgtcgaggcgcggcgagccgcagccattgccttttatggtaatcgtgcgagagggcgcagggacttcctttgtcccaaatctggcggagccgaaatctgggaggcgccgccgcaccccctctagcgggcgcgggcgaagcggtgcggcgccggcaggaaggaaatgggcggggagggccttcgtgcgtcgccgcgccgccgtccccttctccatctccagcctcggggctgccgcagggggacggctgccttcgggggggacggggcagggcggggttcggcttctggcgtgtgaccggcggctctagagcctctgctaaccatgttcatgccttcttctttttcctacagctcctgggcaacgtgctggttattgtgctgtctcatcattttggcaaagaattctaatacgactcactatagggagacccaagctggctagccaaagcttccaccatggcggggctctggctggggctcgtgtggcagaagctgctgctgtggggcgcggcgagtgccctttccctggccggcgccagtctggtcctgagcctgctgcagagggtggcgagctacgcgcggaaatggcagcagatgcggcccatccccacggtggcccgcgcctacccactggtgggccacgcgctgctgatgaagccggacgggcgagaattttttcagcagatcattgagtacacagaggaataccgccacatgccgctgctgaagctctgggtcgggccagtgcccatggtggccctttataatgcagaaaatgtggaggtaattttaactagttcaaagcaaattgacaaatcctctatgtacaagtttttagaaccatggcttggcctaggacttcttacaagtactggaaacaaatggcgctccaggagaaagatgttaacacccactttccattttaccattctggaagatttcttagatatcatgaatgaacaagcaaatatattggttaagaaacttgaaaaacacattaaccaagaagcatttaactgctttttttacatcactctttgtgccttagatatcatctgtgaaacagctatggggaagaatattggtgctcaaagtaatgatgattccgagtatgtccgtgcagtttatagaatgagtgagatgatatttcgaagaataaagatgccctggctttggcttgatctctggtaccttatgtttaaagaaggatgggaacacaaaaagagccttaagatcctacatacttttaccaacagtgtcatcgcggaacgggccaatgaaatgaacgccaatgaagactgtagaggtgatggcaggggctctgccccctccaaaaataaacgcagggcctttcttgacttgcttttaagtgtgactgatgacgaagggaacaggctaagtcatgaagatattcgagaagaagttgacaccttcatgtttgaggggcacgatacaactgcagctgcaataaactggtccttatacctgttgggttctaacccagaagtccagaaaaaagtggatcatgaattggatgacgtgtttgggaagtctgaccgtcccgctacagtagaagacctgaagaaacttcggtatctggaatgtgttattaaggagacccttcgcctttttccttctgttcctttatttgcccgtagtgttagtgaagattgtgaagtggcaggttacagagttctaaaaggcactgaagccgtcatcattccctatgcattgcacagagatccgagatacttccccaaccccgaggagttccagcctgagcggttcttccccgagaatgcacaagggcgccatccatatgcctacgtgcccttctctgctggccccaggaactgtataggtcaaaagtttgctgtgatggaagaaaagaccattctttcgtgcatcctgaggcacttttggatagaatccaaccagaaaagagaagagcttggtctagaaggacagttgattcttcgtccaagtaatggcatctggatcaagttgaagaggagaaatgcagatgaacgctaagcggccgcaactcgagactctagaggttaatcgataatcaacctctggattacaaaatttgtgaaagattgactggtattcttaactatgttgctccttttacgctatgtggatacgctgctttaatgcctttgtatcatgctattgcttcccgtatggctttcattttctcctccttgtataaatcctggttgctgtctctttatgaggagttgtggcccgttgtcaggcaacgtggcgtggtgtgcactgtgtttgctgacgcaacccccactggttggggcattgccaccacctgtcagctcctttccgggactttcgctttccccctccctattgccacggcggaactcatcgccgcctgccttgcccgctgctggacaggggctcggctgttgggcactgacaattccgtggtgttgtcggggaaatcatcgtcctttccttggctgctcgcctgtgttgccacctggattctgcgcgggacgtccttctgctacgtcccttcggccctcaatccagcggaccttccttcccgcggcctgctgccggctctgcggcctcttccgcgtcttcgccttcgccctcagacgagtcggatctccctttgggccgcctccccgcatcgaaacccgctgactagacgactgtgccttctagttgccagccatctgttgtttgcccctcccccgtgccttccttgaccctggaaggtgccactcccactgtcctttcctaataaaatgaggaaattgcatcgcattgtctgagtaggtgtcattctattctggggggtggggtggggcaggacagcaagggggaggattgggaagacaatagcaggcatgctggggatgcggtgggctctatggccgcgggccgcaggaacccctagtgatggagttggccactccctctctgcgcgctcgctcgctcactgaggccgggcgaccaaaggtcgcccgacgcccgggctttgcccgggcggcctcagtgagcgagcgagcgcgcagctgcctgcagg

SEQ ID NO: 63 - DNA, 4539 bp, synthetic construct
  misc_feature 1..4539: note = Synthetically generated expression construct
  source 1..4539: mol_type = other DNA
cctgcaggcagctgcgcgctcgctcgctcactgaggccgcccgggcaaagcccgggcgtcgggcgacctttggtcgcccggcctcagtgagcgagcgagcgcgcagagagggagtggccaactccatcactaggggttcctgcggcctaaggcaattgagatctcgacattgattattgactagttattaatagtaatcaattacggggtcattagttcatagcccatatatggagttccgcgttacataacttacggtaaatggcccgcctggctgaccgcccaacgacccccgcccattgacgtcaataatgacgtatgttcccatagtaacgccaatagggactttccattgacgtcaatgggtggactatttacggtaaactgcccacttggcagtacatcaagtgtatcatatgccaagtacgccccctattgacgtcaatgacggtaaatggcccgcctggcattatgcccagtacatgaccttatgggactttcctacttggcagtacatctacgtattagtcatcgctattaccatgggtcgaggtgagccccacgttctgcttcactctccccatctcccccccctccccacccccaattttgtatttatttattttttaattattttgtgcagcgatgggggcggggggggggggggcgcgcgccaggcggggcggggcggggcgaggggcggggcggggcgaggcggagaggtgcggcggcagccaatcagagcggcgcgctccgaaagtttccttttatggcgaggcggcggcggcggcggccctataaaaagcgaagcgcgcggcgggcgggagtcgctgcgttgccttcgccccgtgccccgctccgcgccgcctcgcgccgcccgccccggctctgactgaccgcgttactcccacaggtgagcgggcgggacggcccttctcctccgggctgtaattagcgcttggtttaatgacggctcgtttcttttctgtggctgcgtgaaagccttaaagggctccgggagggccctttgtgcgggggggagcggctcggggggtgcgtgcgtgtgtgtgtgcgtggggagcgccgcgtgcggcccgcgctgcccggcggctgtgagcgctgcgggcgcggcgcggggctttgtgcgctccgcgtgtgcgcgaggggagcgcggccgggggcggtgccccgcggtgcgggggggctgcgaggggaacaaaggctgcgtgcggggtgtgtgcgtgggggggtgagcagggggtgtgggcgcggcggtcgggctgtaacccccccctgcacccccctccccgagttgctgagcacggcccggcttcgggtgcggggctccgtgcggggcgtggcgcggggctcgccgtgccgggcggggggtggcggcaggtgggggtgccgggcggggcggggccgcctcgggccggggagggctcgggggaggggcgcggcggccccggagcgccggcggctgtcgaggcgcggcgagccgcagccattgccttttatggtaatcgtgcgagagggcgcagggacttcctttgtcccaaatctggcggagccgaaatctgggaggcgccgccgcaccccctctagcgggcgcgggcgaagcggtgcggcgccggcaggaaggaaatgggcggggagggccttcgtgcgtcgccgcgccgccgtccccttctccatctccagcctcggggctgccgcagggggacggctgccttcgggggggacggggcagggcggggttcggcttctggcgtgtgaccggcggctctagagcctctgctaaccatgttcatgccttcttctttttcctacagctcctgggcaacgtgctggttattgtgctgtctcatcattttggcaaagaattctaatacgactcactatagggagacccaagctggctagccaaagcttccaccatggctggactgtggctgggactggtgtggcagaaactgctgctgtggggggccgcttccgcactgtcactggctggggcttcactggtgctgagcctgctgcagagggtggcctcctacgccagaaagtggcagcagatgaggcccatccctaccgtggccagagcctatccactggtgggacacgcactgctgatgaagcctgacggcagagagttctttcagcagatcatcgagtacacagaggagtataggcacatgccactgctgaagctgtgggtgggacccgtgcctatggtggccctgtacaacgccgagaatgtggaagtgatcctgaccagcagcaagcagatcgataagtctagcatgtataagttcctggagccttggctgggcctgggcctgctgacctctacaggcaacaagtggaggagccggagaaagatgctgaccccaacattccactttacaatcctggaggacttcctggacatcatgaacgagcaggccaatatcctggtgaagaagctggagaagcacatcaaccaggaggcctttaattgcttcttttacatcaccctgtgcgccctggacatcatctgtgagacagctatgggcaagaacatcggcgcccagtctaatgacgatagcgagtacgtgcgggccgtgtatagaatgagcgagatgatctttaggcgcatcaagatgccctggctgtggctggatctgtggtatctgatgttcaaggagggctgggagcacaagaagtccctgcagatcctgcacacctttacaaactctgtgatcgccgagagagccaatgagatgaacgccaatgaggactgtaggggcgatggaaggggcagcgccccttccaagaacaagcggagagccttcctggacctgctgctgagcgtgaccgacgatgagggcaatcgcctgtcccacgaggacatccgggaggaggtggatacattcatgtttgagggacacgacaccacagccgccgccatcaactggtccctgtacctgctgggctctaatccagaggtgcagaagaaggtggatcacgagctggacgacgtgttcggcaagtccgacaggccagcaaccgtggaggatctgaagaagctgagatacctggagtgcgtgatcaaggagacactgcgcctgttcccctctgtgcctctgtttgcccggtccgtgtctgaggactgtgaggtggccggctatcgcgtgctgaagggcaccgaggccgtgatcatcccttacgccctgcaccgggaccccaggtatttccctaacccagaggagtttcagccagagagattctttcccgagaatgcccagggcaggcacccttacgcctatgtgccattctccgccggaccaaggaactgcatcggacagaagtttgccgtgatggaggagaaaaccatcctgtcttgtatcctgagacacttctggatcgagagcaatcagaagagggaggagctgggcctggagggacagctgatcctgcggccaagcaacggcatctggatcaaactgaaaagaaggaacgctgacgagaggtaagcggccgcaactcgagactctagaggttaatcgataatcaacctctggattacaaaatttgtgaaagattgactggtattcttaactatgttgctccttttacgctatgtggatacgctgctttaatgcctttgtatcatgctattgcttcccgtatggctttcattttctcctccttgtataaatcctggttgctgtctctttatgaggagttgtggcccgttgtcaggcaacgtggcgtggtgtgcactgtgtttgctgacgcaacccccactggttggggcattgccaccacctgtcagctcctttccgggactttcgctttccccctccctattgccacggcggaactcatcgccgcctgccttgcccgctgctggacaggggctcggctgttgggcactgacaattccgtggtgttgtcggggaaatcatcgtcctttccttggctgctcgcctgtgttgccacctggattctgcgcgggacgtccttctgctacgtcccttcggccctcaatccagcggaccttccttcccgcggcctgctgccggctctgcggcctcttccgcgtcttcgccttcgccctcagacgagtcggatctccctttgggccgcctccccgcatcgaaacccgctgactagacgactgtgccttctagttgccagccatctgttgtttgcccctcccccgtgccttccttgaccctggaaggtgccactcccactgtcctttcctaataaaatgaggaaattgcatcgcattgtctgagtaggtgtcattctattctggggggtggggtggggcaggacagcaagggggaggattgggaagacaatagcaggcatgctggggatgcggtgggctctatggccgcgggccgcaggaacccctagtgatggagttggccactccctctctgcgcgctcgctcgctcactgaggccgggcgaccaaaggtcgcccgacgcccgggctttgcccgggcggcctcagtgagcgagcgagcgcgcagctgcctgcagg

SEQ ID NO: 64 - DNA, 2403 bp, synthetic construct
  misc_feature 1..2403: note = Synthetically generated expression construct
  source 1..2403: mol_type = other DNA
cctgcaggcagctgcgcgctcgctcgctcactgaggccgcccgggcaaagcccgggcgtcgggcgacctttggtcgcccggcctcagtgagcgagcgagcgcgcagagagggagtggacgcgtaggcctgattggctccggtgcccgtcagtgggcagagcgcacatcgcccacagtccccgagaagttggggggaggggtcggcaattgaaccggtgcctagagaaggtggcgcggggtaaactgggaaagtgatgtcgtgtactggctccgcctttttcccgagggtgggggagaaccgtatataagtgcagtagtcgccgtgaacgttctttttcgcaacgggtttgccgccagaacacaggtgtcgtgacgcgaccaggtatgcatctgcagctctaaggtaaatataaaatttttaagtgtataatgtgttaaactactgattctaattgtttctctcttttagattccaacctttggaactgactgcagggatccaagctttctagagccaccatggctggactgtggctgggactggtgtggcagaaactgctgctgtggggggccgcttccgcactgtcactggctggggcttcactggtgctgagcctgctgcagagggtggcctcctacgccagaaagtggcagcagatgaggcccatccctaccgtggccagagcctatccactggtgggacacgcactgctgatgaagcctgacggcagagagttctttcagcagatcatcgagtacacagaggagtataggcacatgccactgctgaagctgtgggtgggacccgtgcctatggtggccctgtacaacgccgagaatgtggaagtgatcctgaccagcagcaagcagatcgataagtctagcatgtataagttcctggagccttggctgggcctgggcctgctgacctctacaggcaacaagtggaggagccggagaaagatgctgaccccaacattccactttacaatcctggaggacttcctggacatcatgaacgagcaggccaatatcctggtgaagaagctggagaagcacatcaaccaggaggcctttaattgcttcttttacatcaccctgtgcgccctggacatcatctgtgagacagctatgggcaagaacatcggcgcccagtctaatgacgatagcgagtacgtgcgggccgtgtatagaatgagcgagatgatctttaggcgcatcaagatgccctggctgtggctggatctgtggtatctgatgttcaaggagggctgggagcacaagaagtccctgcagatcctgcacacctttacaaactctgtgatcgccgagagagccaatgagatgaacgccaatgaggactgtaggggcgatggaaggggcagcgccccttccaagaacaagcggagagccttcctggacctgctgctgagcgtgaccgacgatgagggcaatcgcctgtcccacgaggacatccgggaggaggtggatacattcatgtttgagggacacgacaccacagccgccgccatcaactggtccctgtacctgctgggctctaatccagaggtgcagaagaaggtggatcacgagctggacgacgtgttcggcaagtccgacaggccagcaaccgtggaggatctgaagaagctgagatacctggagtgcgtgatcaaggagacactgcgcctgttcccctctgtgcctctgtttgcccggtccgtgtctgaggactgtgaggtggccggctatcgcgtgctgaagggcaccgaggccgtgatcatcccttacgccctgcaccgggaccccaggtatttccctaacccagaggagtttcagccagagagattctttcccgagaatgcccagggcaggcacccttacgcctatgtgccattctccgccggaccaaggaactgcatcggacagaagtttgccgtgatggaggagaaaaccatcctgtcttgtatcctgagacacttctggatcgagagcaatcagaagagggaggagctgggcctggagggacagctgatcctgcggccaagcaacggcatctggatcaaactgaaaagaaggaacgctgacgagaggtaaaagcttgaattcctcgaggatccaataaaagatctttattttcattagatctgtgtgttggttttttgtgtgtctagttgccagccatctgttgtttgcccctcccccgtgccttccttgaccctggaaggtgccactcccagtttaaacttaattaagggccgcaggaacccctagtgatggagttggccactccctctctgcgcgctcgctcgctcactgaggccgggcgaccaaaggtcgcccgacgcccgggctttgcccgggcggcctcagtgagcgagcgagcgcgcagctgcctgcagg